European Patent Application EP 4 446 425 A1, published October 16, 2024. Title: METHOD FOR PREDICTING PROGNOSIS OF DOGS WITH LTMPHOMA AFTER CHEMOTHERAPY. Applicant: NATIONAL UNIVERSITY CORPORATION HOKKAIDO UNIVERSITY. Application JP. The sequence listing filed with the application follows.

SEQUENCE LISTING (2 sequences)

SEQ ID NO: 1 - DNA, 150 bp, Canis lupus familiaris
  source 1..150: mol_type = genomic DNA
ctgggttctgcggactttgagacaggccccctctgtctccgagtgggtcggtggctgtgctccccgggactccagacattcggatcggaattcgctggtgcctacaaaatgcttgcaaaaacggttctcttgcaactaaggaagagtaga

SEQ ID NO: 2 - DNA, 150 bp, Canis lupus familiaris
  source 1..150: mol_type = genomic DNA
gcgcgggaacgctgcggagaagtcacacgggctcccgaggactcgcacggactctcggtggagcaggcagccggcccagggcacccgccctcggggccccgggggctcccaccgcacgcgccaggggcaggtgatcgcctttcctgcgta